European Patent Application EP 4 484 447 A2, published January 1, 2025. Title: METHODS OF INHIBITING MASP-2 FOR THE TREATMENT AND/OR PREVENTION OF CORONAVIRUS-INDUCED ACUTE RESPIRATORY DISTRESS SYNDROME. Applicant: Omeros Corporation. Application WO PCT/US2021/021217, filed March 5, 2021. The sequence listing filed with the application follows.

SEQUENCE LISTING (85 sequences)

SEQ ID NO: 1 - DNA, 725 bp, Homo sapiens
  source 1..725: mol_type = genomic DNA
ggccaggccagctggacgggcacaccatgaggctgctgaccctcctgggccttctgtgtggctcggtggccacccccttgggcccgaagtggcctgaacctgtgttcgggcgcctggcatcccccggctttccaggggagtatgccaatgaccaggagcggcgctggaccctgactgcaccccccggctaccgcctgcgcctctacttcacccacttcgacctggagctctcccacctctgcgagtacgacttcgtcaagctgagctcgggggccaaggtgctggccacgctgtgcgggcaggagagcacagacacggagcgggcccctggcaaggacactttctactcgctgggctccagcctggacattaccttccgctccgactactccaacgagaagccgttcacggggttcgaggccttctatgcagccgaggacattgacgagtgccaggtggccccgggagaggcgcccacctgcgaccaccactgccacaaccacctgggcggtttctactgctcctgccgcgcaggctacgtcctgcaccgtaacaagcgcacctgctcagagcagagcctctagcctcccctggagctccggcctgcccagcaggtcagaagccagagccagcctgctggcctcagctccgggttgggctgagatggctgtgccccaactcccattcacccaccatggacccaataataaacctggccccacccc

SEQ ID NO: 2 - protein, 185 aa, Homo sapiens
MRLLTLLGLLCGSVATPLGPKWPEPVFGRLASPGFPGEYANDQERRWTLTAPPGYRLRLYFTHFDLELSHLCEYDFVKLSSGAKVLATLCGQESTDTERAPGKDTFYSLGSSLDITFRSDYSNEKPFTGFEAFYAAEDIDECQVAPGEAPTCDHHCHNHLGGFYCSCRAGYVLHRNKRTCSEQSL

SEQ ID NO: 3 - protein, 170 aa, Homo sapiens
TPLGPKWPEPVFGRLASPGFPGEYANDQERRWTLTAPPGYRLRLYFTHFDLELSHLCEYDFVKLSSGAKVLATLCGQESTDTERAPGKDTFYSLGSSLDITFRSDYSNEKPFTGFEAFYAAEDIDECQVAPGEAPTCDHHCHNHLGGFYCSCRAGYVLHRNKRTCSEQSL

SEQ ID NO: 4 - DNA, 2460 bp, Homo sapiens
  source 1..2460: mol_type = other DNA
ggccagctggacgggcacaccatgaggctgctgaccctcctgggccttctgtgtggctcggtggccacccccttgggcccgaagtggcctgaacctgtgttcgggcgcctggcatcccccggctttccaggggagtatgccaatgaccaggagcggcgctggaccctgactgcaccccccggctaccgcctgcgcctctacttcacccacttcgacctggagctctcccacctctgcgagtacgacttcgtcaagctgagctcgggggccaaggtgctggccacgctgtgcgggcaggagagcacagacacggagcgggcccctggcaaggacactttctactcgctgggctccagcctggacattaccttccgctccgactactccaacgagaagccgttcacggggttcgaggccttctatgcagccgaggacattgacgagtgccaggtggccccgggagaggcgcccacctgcgaccaccactgccacaaccacctgggcggtttctactgctcctgccgcgcaggctacgtcctgcaccgtaacaagcgcacctgctcagccctgtgctccggccaggtcttcacccagaggtctggggagctcagcagccctgaatacccacggccgtatcccaaactctccagttgcacttacagcatcagcctggaggaggggttcagtgtcattctggactttgtggagtccttcgatgtggagacacaccctgaaaccctgtgtccctacgactttctcaagattcaaacagacagagaagaacatggcccattctgtgggaagacattgccccacaggattgaaacaaaaagcaacacggtgaccatcacctttgtcacagatgaatcaggagaccacacaggctggaagatccactacacgagcacagcgcagccttgcccttatccgatggcgccacctaatggccacgtttcacctgtgcaagccaaatacatcctgaaagacagcttctccatcttttgcgagactggctatgagcttctgcaaggtcacttgcccctgaaatcctttactgcagtttgtcagaaagatggatcttgggaccggccaatgcccgcgtgcagcattgttgactgtggccctcctgatgatctacccagtggccgagtggagtacatcacaggtcctggagtgaccacctacaaagctgtgattcagtacagctgtgaagagaccttctacacaatgaaagtgaatgatggtaaatatgtgtgtgaggctgatggattctggacgagctccaaaggagaaaaatcactcccagtctgtgagcctgtttgtggactatcagcccgcacaacaggagggcgtatatatggagggcaaaaggcaaaacctggtgattttccttggcaagtcctgatattaggtggaaccacagcagcaggtgcacttttatatgacaactgggtcctaacagctgctcatgccgtctatgagcaaaaacatgatgcatccgccctggacattcgaatgggcaccctgaaaagactatcacctcattatacacaagcctggtctgaagctgtttttatacatgaaggttatactcatgatgctggctttgacaatgacatagcactgattaaattgaataacaaagttgtaatcaatagcaacatcacgcctatttgtctgccaagaaaagaagctgaatcctttatgaggacagatgacattggaactgcatctggatggggattaacccaaaggggttttcttgctagaaatctaatgtatgtcgacataccgattgttgaccatcaaaaatgtactgctgcatatgaaaagccaccctatccaaggggaagtgtaactgctaacatgctttgtgctggcttagaaagtgggggcaaggacagctgcagaggtgacagcggaggggcactggtgtttctagatagtgaaacagagaggtggtttgtgggaggaatagtgtcctggggttccatgaattgtggggaagcaggtcagtatggagtctacacaaaagttattaactatattccctggatcgagaacataattagtgatttttaacttgcgtgtctgcagtcaaggattcttcatttttagaaatgcctgtgaagaccttggcagcgacgtggctcgagaagcattcatcattactgtggacatggcagttgttgctccacccaaaaaaacagactccaggtgaggctgctgtcatttctccacttgccagtttaattccagccttacccattgactcaaggggacataaaccacgagagtgacagtcatctttgcccacccagtgtaatgtcactgctcaaattacatttcattaccttaaaaagccagtctcttttcatactggctgttggcatttctgtaaactgcctgtccatgctctttgtttttaaacttgttcttattgaaaaaaaaaaaaaaaaa

SEQ ID NO: 5 - protein, 686 aa, Homo sapiens
MRLLTLLGLLCGSVATPLGPKWPEPVFGRLASPGFPGEYANDQERRWTLTAPPGYRLRLYFTHFDLELSHLCEYDFVKLSSGAKVLATLCGQESTDTERAPGKDTFYSLGSSLDITFRSDYSNEKPFTGFEAFYAAEDIDECQVAPGEAPTCDHHCHNHLGGFYCSCRAGYVLHRNKRTCSALCSGQVFTQRSGELSSPEYPRPYPKLSSCTYSISLEEGFSVILDFVESFDVETHPETLCPYDFLKIQTDREEHGPFCGKTLPHRIETKSNTVTITFVTDESGDHTGWKIHYTSTAQPCPYPMAPPNGHVSPVQAKYILKDSFSIFCETGYELLQGHLPLKSFTAVCQKDGSWDRPMPACSIVDCGPPDDLPSGRVEYITGPGVTTYKAVIQYSCEETFYTMKVNDGKYVCEADGFWTSSKGEKSLPVCEPVCGLSARTTGGRIYGGQKAKPGDFPWQVLILGGTTAAGALLYDNWVLTAAHAVYEQKHDASALDIRMGTLKRLSPHYTQAWSEAVFIHEGYTHDAGFDNDIALIKLNNKVVINSNITPICLPRKEAESFMRTDDIGTASGWGLTQRGFLARNLMYVDIPIVDHQKCTAAYEKPPYPRGSVTANMLCAGLESGGKDSCRGDSGGALVFLDSETERWFVGGIVSWGSMNCGEAGQYGVYTKVINYIPWIENIISDF

SEQ ID NO: 6 - protein, 671 aa, Homo sapiens
TPLGPKWPEPVFGRLASPGFPGEYANDQERRWTLTAPPGYRLRLYFTHFDLELSHLCEYDFVKLSSGAKVLATLCGQESTDTERAPGKDTFYSLGSSLDITFRSDYSNEKPFTGFEAFYAAEDIDECQVAPGEAPTCDHHCHNHLGGFYCSCRAGYVLHRNKRTCSALCSGQVFTQRSGELSSPEYPRPYPKLSSCTYSISLEEGFSVILDFVESFDVETHPETLCPYDFLKIQTDREEHGPFCGKTLPHRIETKSNTVTITFVTDESGDHTGWKIHYTSTAQPCPYPMAPPNGHVSPVQAKYILKDSFSIFCETGYELLQGHLPLKSFTAVCQKDGSWDRPMPACSIVDCGPPDDLPSGRVEYITGPGVTTYKAVIQYSCEETFYTMKVNDGKYVCEADGFWTSSKGEKSLPVCEPVCGLSARTTGGRIYGGQKAKPGDFPWQVLILGGTTAAGALLYDNWVLTAAHAVYEQKHDASALDIRMGTLKRLSPHYTQAWSEAVFIHEGYTHDAGFDNDIALIKLNNKVVINSNITPICLPRKEAESFMRTDDIGTASGWGLTQRGFLARNLMYVDIPIVDHQKCTAAYEKPPYPRGSVTANMLCAGLESGGKDSCRGDSGGALVFLDSETERWFVGGIVSWGSMNCGEAGQYGVYTKVINYIPWIENIISDF

SEQ ID NO: 7 - DNA, 4900 bp, Homo sapiens
  source 1..4900: mol_type = genomic DNA
cctgtcctgcctgcctggaactctgagcaggctggagtcatggagtcgattcccagaatcccagagtcagggaggctgggggcaggggcaggtcactggacaaacagatcaaaggtgagaccagcgtaggactgcagaccaggccaggccagctggacgggcacaccatgaggtaggtgggcgccacagcctccctgcagggtgtggggtgggagcacaggcctgggcctcaccgcccctgccctgcccataggctgctgaccctcctgggccttctgtgtggctcggtggccacccccttaggcccgaagtggcctgaacctgtgttcgggcgcctggcatcccccggctttccaggggagtatgccaatgaccaggagcggcgctggaccctgactgcaccccccggctaccgcctgcgcctctacttcacccacttcgacctggagctctcccacctctgcgagtacgacttcgtcaaggtgccgtcagacgggagggctggggtttctcagggtcggggggtccccaaggagtagccagggttcagggacacctgggagcaggggccaggcttggccaggagggagatcaggcctgggtcttgccttcactccctgtgacacctgaccccacagctgagctcgggggccaaggtgctggccacgctgtgcgggcaggagagcacagacacggagcgggcccctggcaaggacactttctactcgctgggctccagcctggacattaccttccgctccgactactccaacgagaagccgttcacggggttcgaggccttctatgcagccgagggtgagccaagaggggtcctgcaacatctcagtctgcgcagctggctgtgggggtaactctgtcttaggccaggcagccctgccttcagtttccccacctttcccagggcaggggagaggcctctggcctgacatcatccacaatgcaaagaccaaaacagccgtgacctccattcacatgggctgagtgccaactctgagccagggatctgaggacagcatcgcctcaagtgacgcagggactggccgggcgcggcagctcacgcctgtaattccagcactttgggaggccgaggctggcttgataatttgagggtcaggagttcaaggccagccagggcaacacggtgaaactctatctccactaaaactacaaaaattagctgggcgtggtggtgcgcacctggaatcccagctactagggaggctgaggcaggagaattgcttgaacctgcgaggtggaggctgcagtgaacagagattgcaccactacactccacctgggcgacagactagactccgtctcaaaaaacaaaaaacaaaaaccacgcagggccgagggcccatttacaagctgacaaagtgggccctgccagcgggagcgctgcaggatgtttgattttcagatcccagtccctgcagagaccaactgtgtgacctctggcaagtggctcaatttctctgctccttagaagctgctgcaagggttcagcgctgtagccccgccccctgggtttgattgactcccctcattagctgggtgacctcggccggacactgaaactcccactggtttaacagaggtgatgtttgcatctttctcccagcgctgctgggagcttgcagcgaccctaggcctgtaaggtgattggcccggcaccagtcccgcaccctagacaggacctaggcctcctctgaggtccactctgaggtcatggatctcctgggaggagtccaggctggatcccgcctctttccctcctgacggcctgcctggccctgcctctcccccagacattgacgagtgccaggtggccccgggagaggcgcccacctgcgaccaccactgccacaaccacctgggcggtttctactgctcctgccgcgcaggctacgtcctgcaccgtaacaagcgcacctgctcaggtgagggaggctgcctgggccccaacgcaccctctcctgggatacccggggctcctcagggccattgctgctctgcccaggggtgcggagggcctgggcctggacactgggtgcttctaggccctgctgcctccagctccccttctcagccctgcttcccctctcagcagccaggctcatcagtgccaccctgccctagcactgagactaattctaacatcccactgtgtacctggttccacctgggctctgggaacccctcatgtagccacgggagagtcggggtatctaccctcgttccttggactgggttcctgttccctgcactgggggacgggccagtgctctggggcgtgggcagccccaccctgtggcgctgaccctgctcccccgactcggtttctcctctcggggtctctccttgcctctctgatctctcttccagagcagagcctctagcctcccctggagctccggctgcccagcaggtcagaagccagagccaggctgctggcctcagctccgggttgggctgagatgctgtgccccaactcccattcacccaccatggacccaataataaacctggccccaccccacctgctgccgcgtgtctctggggtgggagggtcgggaggcggtggggcgcgctcctctctgcctaccctcctcacagcctcatgaaccccaggtctgtgggagcctcctccatggggccacacggtccttggcctcaccccctgttttgaagatggggcactgaggccggagaggggtaaggcctcgctcgagtccaggtccccagaggctgagcccagagtaatcttgaaccacccccattcagggtctggcctggaggagcctgacccacagaggagacaccctgggagatattcattgaggggtaatctggtcccccgcaaatccaggggtgattcccactgccccataggcacagccacgtggaagaaggcaggcaatgttggggctcctcacttcctagaggcctcacaactcaaatgccccccactgcagctgggggtggggtggtggtatgggatggggaccaagccttccttgaaggatagagcccagcccaacaccccgccccgtggcagcagcatcacgtgttccagcgaggaaggagagcaccagactcagtcatgatcactgttgccttgaacttccaagaacagccccagggcaagggtcaaaacaggggaaagggggtgatgagagatccttcttccggatgttcctccaggaaccagggggctggctggtcttggctgggttcgggtaggagacccatgatgaataaacttgggaatcactggggtggctgtaagggaatttaggggagctccgaaggggcccttaggctcgaggagatgctcctctcttttcccgaattcccagggacccaggagagtgtcccttcttcctcttcctgtgtgtccatccacccccgccccccgccctggcagagctggtggaactcagtgctctagcccctaccctggggttgcgactctggctcaggacaccaccacgctccctgggggtgtgagtgagggcctgtgcgctccatcccgagtgctgcctgtttcagctaaagcctcaaagcaagagaaaccccctctctaagcggcccctcagccatcgggtgggtcgtttggtttctgggtaggcctcaggggctggccacctgcagggcccagcccaacccagggatgcagatgtcccagccacatccctgtcccagtttcctgctccccaaggcatccaccctgctgttggtgcgagggctgatagagggcacgccaagtcactcccctgcccttccctccttccagccctgtgctccggccaggtcttcacccagaggtctggggagctcagcagccctgaatacccacggccgtatcccaaactctccagttgcacttacagcatcagcctggaggaggggttcagtgtcattctggactttgtggagtccttcgatgtggagacacaccctgaaaccctgtgtccctacgactttctcaaggtctggctcctgggcccctcatcttgtcccagatcctcccccttcagcccagctgcaccccctacttcctgcagcatggcccccaccacgttcccgtcaccctcggtgaccccacctcttcaggtgctctatggaggtcaaggctggggcttcgagtacaagtgtgggaggcagagtggggaggggcaccccaatccatggcctgggttggcctcattggctgtccctgaaatgctgaggaggtgggttacttccctccgcccaggccagacccaggcagctgctccccagctttcatgagcttctttctcagattcaaacagacagagaagaacatggcccattctgtgggaagacattgccccacaggattgaaacaaaaagcaacacggtgaccatcacctttgtcacagatgaatcaggagaccacacaggctggaagatccactacacgagcacagtgagcaagtgggctcagatccttggtggaagcgcagagctgcctctctctggagtgcaaggagctgtagagtgtagggctcttctgggcaggactaggaagggacaccaggtttagtggtgctgaggtctgaggcagcagcttctaaggggaagcacccgtgccctcctcagcagcacccagcatcttcaccactcattcttcaaccacccattcacccatcactcatcttttacccacccaccctttgccactcatccttctgtccctcatccttccaaccattcatcaatcacccacccatccatcctttgccacacaaccatccacccattcttctacctacccatcctatccatccatccttctatcagcatccttctaccacccatccttcgttcggtcatccatcatcatccatccatc

SEQ ID NO: 8 - protein, 136 aa, Homo sapiens
MRLLTLLGLLCGSVATPLGPKWPEPVFGRLASPGFPGEYANDQERRWTLTAPPGYRLRLYFTHFDLELSHLCEYDFVKLSSGAKVLATLCGQESTDTERAPGKDTFYSLGSSLDITFRSDYSNEKPFTGFEAFYAA

SEQ ID NO: 9 - protein, 181 aa, Homo sapiens
MRLLTLLGLLCGSVATPLGPKWPEPVFGRLASPGFPGEYANDQERRWTLTAPPGYRLRLYFTHFDLELSHLCEYDFVKLSSGAKVLATLCGQESTDTERAPGKDTFYSLGSSLDITFRSDYSNEKPFTGFEAFYAAEDIDECQVAPGEAPTCDHHCHNHLGGFYCSCRAGYVLHRNKRTCS

SEQ ID NO: 10 - protein, 293 aa, Homo sapiens
MRLLTLLGLLCGSVATPLGPKWPEPVFGRLASPGFPGEYANDQERRWTLTAPPGYRLRLYFTHFDLELSHLCEYDFVKLSSGAKVLATLCGQESTDTERAPGKDTFYSLGSSLDITFRSDYSNEKPFTGFEAFYAAEDIDECQVAPGEAPTCDHHCHNHLGGFYCSCRAGYVLHRNKRTCSALCSGQVFTQRSGELSSPEYPRPYPKLSSCTYSISLEEGFSVILDFVESFDVETHPETLCPYDFLKIQTDREEHGPFCGKTLPHRIETKSNTVTITFVTDESGDHTGWKIHY

SEQ ID NO: 11 - protein, 41 aa, Homo sapiens
EDIDECQVAPGEAPTCDHHCHNHLGGFYCSCRAGYVLHRNK

SEQ ID NO: 12 - protein, 242 aa, Homo sapiens
IYGGQKAKPGDFPWQVLILGGTTAAGALLYDNWVLTAAHAVYEQKHDASALDIRMGTLKRLSPHYTQAWSEAVFIHEGYTHDAGFDNDIALIKLNNKVVINSNITPICLPRKEAESFMRTDDIGTASGWGLTQRGFLARNLMYVDIPIVDHQKCTAAYEKPPYPRGSVTANMLCAGLESGGKDSCRGDSGGALVFLDSETERWFVGGIVSWGSMNCGEAGQYGVYTKVINYIPWIENIISDF

SEQ ID NO: 13 - protein, 16 aa, synthetic construct
  REGION 1..16: note = Synthetic
GKDSCRGDAGGALVFL

SEQ ID NO: 14 - protein, 15 aa, synthetic construct
  REGION 1..15: note = Synthetic
TPLGPKWPEPVFGRL

SEQ ID NO: 15 - protein, 43 aa, synthetic construct
  REGION 1..43: note = Synthetic
TAPPGYRLRLYFTHFDLELSHLCEYDFVKLSSGAKVLATLCGQ

SEQ ID NO: 16 - protein, 8 aa, synthetic construct
  REGION 1..8: note = Synthetic
TFRSDYSN

SEQ ID NO: 17 - protein, 25 aa, synthetic construct
  REGION 1..25: note = Synthetic
FYSLGSSLDITFRSDYSNEKPFTGF

SEQ ID NO: 18 - protein, 9 aa, synthetic construct
  REGION 1..9: note = Synthetic
IDECQVAPG

SEQ ID NO: 19 - protein, 25 aa, synthetic construct
  REGION 1..25: note = Synthetic
ANMLCAGLESGGKDSCRGDSGGALV

SEQ ID NO: 20 - DNA, 960 bp, Homo sapiens
  source 1..960: mol_type = other DNA
attaactgagattaaccttccctgagttttctcacaccaaggtgaggaccatgtccctgtttccatcactccctctccttctcctgagtatggtggcagcgtcttactcagaaactgtgacctgtgaggatgcccaaaagacctgccctgcagtgattgcctgtagctctccaggcatcaacggcttcccaggcaaagatgggcgtgatggcaccaagggagaaaagggggaaccaggccaagggctcagaggcttacagggcccccctggaaagttggggcctccaggaaatccagggccttctgggtcaccaggaccaaagggccaaaaaggagaccctggaaaaagtccggatggtgatagtagcctggctgcctcagaaagaaaagctctgcaaacagaaatggcacgtatcaaaaagtggctcaccttctctctgggcaaacaagttgggaacaagttcttcctgaccaatggtgaaataatgacctttgaaaaagtgaaggccttgtgtgtcaagttccaggcctctgtggccacccccaggaatgctgcagagaatggagccattcagaatctcatcaaggaggaagccttcctgggcatcactgatgagaagacagaagggcagtttgtggatctgacaggaaatagactgacctacacaaactggaacgagggtgaacccaacaatgctggttctgatgaagattgtgtattgctactgaaaaatggccagtggaatgacgtcccctgctccacctcccatctggccgtctgtgagttccctatctgaagggtcatatcactcaggccctccttgtctttttactgcaacccacaggcccacagtatgcttgaaaagataaattatatcaatttcctcatatccagtattgttccttttgtgggcaatcactaaaaatgatcactaacagcaccaacaaagcaataatagt

SEQ ID NO: 21 - protein, 248 aa, Homo sapiens
MSLFPSLPLLLLSMVAASYSETVTCEDAQKTCPAVIACSSPGINGFPGKDGRDGTKGEKGEPGQGLRGLQGPPGKLGPPGNPGPSGSPGPKGQKGDPGKSPDGDSSLAASERKALQTEMARIKKWLTFSLGKQVGNKFFLTNGEIMTFEKVKALCVKFQASVATPRNAAENGAIQNLIKEEAFLGITDEKTEGQFVDLTGNRLTYTNWNEGEPNNAGSDEDCVLLLKNGQWNDVPCSTSHLAVCEFPI

SEQ ID NO: 22 - protein, 6 aa, synthetic construct
  REGION 1..6: note = Synthetic
  SITE 1: note = MISC_FEATURE - Wherein X at position 1 represents hydroxyproline
  SITE 4: note = MISC_FEATURE - Wherein X at position 4 represents hydrophobic residue
XGKXGP

SEQ ID NO: 23 - protein, 5 aa, synthetic construct
  REGION 1..5: note = Synthetic
  SITE 1: note = MISC_FEATURE - Wherein X represents hydroxyproline
XGKLG

SEQ ID NO: 24 - protein, 16 aa, synthetic construct
  REGION 1..16: note = Synthetic
  REGION 9..15: note = MISC_FEATURE - Wherein X at positions 9 and 15 represents hydroxyproline
GLRGLQGPXGKLGPXG

SEQ ID NO: 25 - protein, 27 aa, synthetic construct
  REGION 1..27: note = Synthetic
  REGION 3..27: note = MISC_FEATURE - Wherein X at positions 3, 6, 15, 21, 24, 27 representshydroxyproline
GPXGPXGLRGLQGPXGKLGPXGPXGPX

SEQ ID NO: 26 - protein, 53 aa, synthetic construct
  REGION 1..53: note = Synthetic
  SITE 26: note = misc_feature - Xaa can be any naturally occurring amino acid
  SITE 32: note = misc_feature - Xaa can be any naturally occurring amino acid
  SITE 35: note = misc_feature - Xaa can be any naturally occurring amino acid
  SITE 41: note = misc_feature - Xaa can be any naturally occurring amino acid
  SITE 50: note = misc_feature - Xaa can be any naturally occurring amino acid
GKDGRDGTKGEKGEPGQGLRGLQGPXGKLGPXGNXGPSGSXGPKGQKGDXGKS

SEQ ID NO: 27 - protein, 33 aa, synthetic construct
  REGION 1..33: note = Synthetic
  REGION 3..33: note = MISC_FEATURE - Wherein X at positions 3, 6, 12, 18, 21, 30, 33 representshydroxyproline
GAXGSXGEKGAXGPQGPXGPXGKMGPKGEXGDX

SEQ ID NO: 28 - protein, 45 aa, synthetic construct
  REGION 1..45: note = Synthetic
  REGION 3..45: note = MISC_FEATURE - Wherein X at positions 3, 6, 9, 27, 30, 36, 42, 45 representshydroxyproline
GCXGLXGAXGDKGEAGTNGKRGERGPXGPXGKAGPXGPNGAXGEX

SEQ ID NO: 29 - protein, 24 aa, synthetic construct
  REGION 1..24: note = Synthetic
LQRALEILPNRVTIKANRPFLVFI

SEQ ID NO: 30 - DNA, 559 bp, Homo sapiens
  source 1..559: mol_type = other DNA
atgaggctgctgaccctcctgggccttctgtgtggctcggtggccacccccttgggcccgaagtggcctgaacctgtgttcgggcgcctggcatcccccggctttccaggggagtatgccaatgaccaggagcggcgctggaccctgactgcaccccccggctaccgcctgcgcctctacttcacccacttcgacctggagctctcccacctctgcgagtacgacttcgtcaagctgagctcgggggccaaggtgctggccacgctgtgcgggcaggagagcacagacacggagcgggcccctggcaaggacactttctactcgctgggctccagcctggacattaccttccgctccgactactccaacgagaagccgttcacggggttcgaggccttctatgcagccgaggacattgacgagtgccaggtggccccgggagaggcgcccacctgcgaccaccactgccacaaccacctgggcggtttctactgctcctgccgcgcaggctacgtcctgcaccgtaacaagcgcacctgctcagccctgtgctccggcc

SEQ ID NO: 31 - DNA, 34 bp, synthetic construct
  misc_feature 1..34: note = Synthetic
  source 1..34: mol_type = other DNA
cgggcacaccatgaggctgctgaccctcctgggc

SEQ ID NO: 32 - DNA, 33 bp, synthetic construct
  misc_feature 1..33: note = Synthetic
  source 1..33: mol_type = other DNA
gacattaccttccgctccgactccaacgagaag

SEQ ID NO: 33 - DNA, 33 bp, synthetic construct
  misc_feature 1..33: note = Synthetic
  source 1..33: mol_type = other DNA
agcagccctgaatacccacggccgtatcccaaa

SEQ ID NO: 34 - DNA, 26 bp, synthetic construct
  misc_feature 1..26: note = Synthetic
  source 1..26: mol_type = other DNA
cgggatccatgaggctgctgaccctc

SEQ ID NO: 35 - DNA, 19 bp, synthetic construct
  misc_feature 1..19: note = Synthetic
  source 1..19: mol_type = other DNA
ggaattcctaggctgcata

SEQ ID NO: 36 - DNA, 19 bp, synthetic construct
  misc_feature 1..19: note = Synthetic
  source 1..19: mol_type = other DNA
ggaattcctacagggcgct

SEQ ID NO: 37 - DNA, 19 bp, synthetic construct
  misc_feature 1..19: note = Synthetic
  source 1..19: mol_type = other DNA
ggaattcctagtagtggat

SEQ ID NO: 38 - DNA, 25 bp, synthetic construct
  misc_feature 1..25: note = Synthetic
  source 1..25: mol_type = other DNA
tgcggccgctgtaggtgctgtcttt

SEQ ID NO: 39 - DNA, 23 bp, synthetic construct
  misc_feature 1..23: note = Synthetic
  source 1..23: mol_type = other DNA
ggaattcactcgttattctcgga

SEQ ID NO: 40 - DNA, 17 bp, synthetic construct
  misc_feature 1..17: note = Synthetic
  source 1..17: mol_type = other DNA
tccgagaataacgagtg

SEQ ID NO: 41 - DNA, 29 bp, synthetic construct
  misc_feature 1..29: note = Synthetic
  source 1..29: mol_type = other DNA
cattgaaagctttggggtagaagttgttc

SEQ ID NO: 42 - DNA, 27 bp, synthetic construct
  misc_feature 1..27: note = Synthetic
  source 1..27: mol_type = other DNA
cgcggccgcagctgctcagagtgtaga

SEQ ID NO: 43 - DNA, 28 bp, synthetic construct
  misc_feature 1..28: note = Synthetic
  source 1..28: mol_type = other DNA
cggtaagcttcactggctcagggaaata

SEQ ID NO: 44 - DNA, 37 bp, synthetic construct
  misc_feature 1..37: note = Synthetic
  source 1..37: mol_type = other DNA
aagaagcttgccgccaccatggattggctgtggaact

SEQ ID NO: 45 - DNA, 31 bp, synthetic construct
  misc_feature 1..31: note = Synthetic
  source 1..31: mol_type = other DNA
cgggatcctcaaactttcttgtccaccttgg

SEQ ID NO: 46 - DNA, 36 bp, synthetic construct
  misc_feature 1..36: note = Synthetic
  source 1..36: mol_type = other DNA
aagaaagcttgccgccaccatgttctcactagctct

SEQ ID NO: 47 - DNA, 26 bp, synthetic construct
  misc_feature 1..26: note = Synthetic
  source 1..26: mol_type = other DNA
cgggatccttctccctctaacactct

SEQ ID NO: 48 - protein, 9 aa, synthetic construct
  REGION 1..9: note = Synthetic
EPKSCDKTH

SEQ ID NO: 49 - DNA, 4960 bp, Homo Sapiens
  source 1..4960: mol_type = genomic DNA
ccggacgtggtggcgcatgcctgtaatcccagctactcgggaggctgaggcaggagaattgctcgaaccccggaggcagaggtttggtggctcacacctgtaatcccagcactttgcgaggctgaggcaggtgcatcgctttggctcaggagttcaagaccagcctgggcaacacagggagacccccatctctacaaaaaacaaaaacaaatataaaggggataaaaaaaaaaaaaagacaagacatgaatccatgaggacagagtgtggaagaggaagcagcagcctcaaagttctggaagctggaagaacagataaacaggtgtgaaataactgcctggaaagcaacttctttttttttttttttttttttgaggtggagtctcactctgtcgtccaggctggagtgcagtggtgcgatctcggatcactgcaacctccgcctcccaggctcaagcaattctcctgcctcagcctcccgagtagctgggattataagtgcgcgctgccacacctggatgatttttgtatttttagtagagatgggatttcaccatgttggtcaggctggtctcaaactcccaacctcgtgatccacccaccttggcctcccaaagtgctgggattacaggtataagccaccgagcccagccaaaagcgacttctaagcctgcaagggaatcgggaattggtggcaccaggtccttctgacagggtttaagaaattagccagcctgaggctgggcacggtggctcacacctgtaatcccagcactttgggaggctaaggcaggtggatcacctgagggcaggagttcaagaccagcctgaccaacatggagaaaccccatccctaccaaaaataaaaaattagccaggtgtggtggtgctcgcctgtaatcccagctacttgggaggctgaggtgggaggattgcttgaacacaggaagtagaggctgcagtgagctatgattgcagcactgcactgaagccggggcaacagaacaagatccaaaaaaaagggaggggtgaggggcagagccaggatttgtttccaggctgttgttacctaggtccgactcctggctcccagagcagcctgtcctgcctgcctggaactctgagcaggctggagtcatggagtcgattcccagaatcccagagtcagggaggctgggggcaggggcaggtcactggacaaacagatcaaaggtgagaccagcgtagggctgcagaccaggccaggccagctggacgggcacaccatgaggtaggtgggcgcccacagcctccctgcagggtgtggggtgggagcacaggcctgggccctcaccgcccctgccctgcccataggctgctgaccctcctgggccttctgtgtggctcggtggccacccccttgggcccgaagtggcctgaacctgtgttcgggcgcctggcatcccccggctttccaggggagtatgccaatgaccaggagcggcgctggaccctgactgcaccccccggctaccgcctgcgcctctacttcacccacttcgacctggagctctcccacctctgcgagtacgacttcgtcaaggtgccgtcaggacgggagggctggggtttctcagggtcggggggtccccaaggagtagccagggttcagggacacctgggagcaggggccaggcttggccaggagggagatcaggcctgggtcttgccttcactccctgtgacacctgaccccacagctgagctcgggggccaaggtgctggccacgctgtgcgggcaggagagcacagacacggagcgggcccctggcaaggacactttctactcgctgggctccagcctggacattaccttccgctccgactactccaacgagaagccgttcacggggttcgaggccttctatgcagccgagggtgagccaagaggggtcctgcaacatctcagtctgcgcagctggctgtgggggtaactctgtcttaggccaggcagccctgccttcagtttccccacctttcccagggcaggggagaggcctctggcctgacatcatccacaatgcaaagaccaaaacagccgtgacctccattcacatgggctgagtgccaactctgagccagggatctgaggacagcatcgcctcaagtgacgcagggactggccgggcgcagcagctcacgcctgtaattccagcactttgggaggccgaggctggctgatcatttgaggtcaggagttcaaggccagccagggcaacacggtgaaactctatctccactaaaactacaaaaattagctgggcgtggtggtgcgcacctggaatcccagctactagggaggctgaggcaggagaattgcttgaacctgcgaggtggaggctgcagtgaacagagattgcaccactacactccagcctgggcgacagagctagactccgtctcaaaaaacaaaaaacaaaaacgacgcaggggccgagggccccatttacagctgacaaagtggggccctgccagcgggagcgctgccaggatgtttgatttcagatcccagtccctgcagagaccaactgtgtgacctctggcaagtggctcaatttctctgctccttaggaagctgctgcaagggttcagcgctgtagccccgccccctgggtttgattgactcccctcattagctgggtgacctcgggccggacactgaaactcccactggtttaacagaggtgatgtttgcatctttctcccagcgctgctgggagcttgcagcgaccctaggcctgtaaggtgattggcccggcaccagtcccgcaccctagacaggacgaggcctcctctgaggtccactctgaggtcatggatctcctgggaggagtccaggctggatcccgcctctttccctcctgacggcctgcctggccctgcctctcccccagacattgacgagtgccaggtggccccgggagaggcgcccacctgcgaccaccactgccacaaccacctgggcggtttctactgctcctgccgcgcaggctacgtcctgcaccgtaacaagcgcacctgctcagccctgtgctccggccaggtcttcacccagaggtctggggagctcagcagccctgaatacccacggccgtatcccaaactctccagttgcacttacagcatcagcctggaggaggggttcagtgtcattctggactttgtggagtccttcgatgtggagacacaccctgaaaccctgtgtccctacgactttctcaagattcaaacagacagagaagaacatggcccattctgtgggaagacattgccccacaggattgaaacaaaaagcaacacggtgaccatcacctttgtcacagatgaatcaggagaccacacaggctggaagatccactacacgagcacagcgcacgcttgcccttatccgatggcgccacctaatggccacgtttcacctgtgcaagccaaatacatcctgaaagacagcttctccatcttttgcgagactggctatgagcttctgcaaggtcacttgcccctgaaatcctttactgcagtttgtcagaaagatggatcttgggaccggccaatgcccgcgtgcagcattgttgactgtggccctcctgatgatctacccagtggccgagtggagtacatcacaggtcctggagtgaccacctacaaagctgtgattcagtacagctgtgaagagaccttctacacaatgaaagtgaatgatggtaaatatgtgtgtgaggctgatggattctggacgagctccaaaggagaaaaatcactcccagtctgtgagcctgtttgtggactatcagcccgcacaacaggagggcgtatatatggagggcaaaaggcaaaacctggtgattttccttggcaagtcctgatattaggtggaaccacagcagcaggtgcacttttatatgacaactgggtcctaacagctgctcatgccgtctatgagcaaaaacatgatgcatccgccctggacattcgaatgggcaccctgaaaagactatcacctcattatacacaagcctggtctgaagctgtttttatacatgaaggttatactcatgatgctggctttgacaatgacatagcactgattaaattgaataacaaagttgtaatcaatagcaacatcacgcctatttgtctgccaagaaaagaagctgaatcctttatgaggacagatgacattggaactgcatctggatggggattaacccaaaggggttttcttgctagaaatctaatgtatgtcgacataccgattgttgaccatcaaaaatgtactgctgcatatgaaaagccaccctatccaaggggaagtgtaactgctaacatgctttgtgctggcttagaaagtgggggcaaggacagctgcagaggtgacagcggaggggcactggtgtttctagatagtgaaacagagaggtggtttgtgggaggaatagtgtcctggggttccatgaattgtggggaagcaggtcagtatggagtctacacaaaagttattaactatattccctggatcgagaacataattagtgatttttaacttgcgtgtctgcagtcaaggattcttcatttttagaaatgcctgtgaagaccttggcagcgacgtggctcgagaagcattcatcattactgtggacatggcagttgttgctccacccaaaaaaacagactccaggtgaggctgctgtcatttctccacttgccagtttaattccagccttacccattgactcaaggggacataaaccacgagagtgacagtcatctttgcccacccagtgtaatgtcactgctcaaattacatttcattaccttaaaaagccagtctcttttcatactggctgttggcatttctgtaaactgcctgtccatgctctttgtttttaaacttgttcttattgaaaaaaaaaaaaaaaaa

SEQ ID NO: 50 - DNA, 2090 bp, Murine
  source 1..2090: mol_type = other DNA
ggcgctggactgcagagctatggtggcacaccatgaggctactcatcttcctgggtctgctgtggagtttggtggccacacttctgggttcaaagtggcctgaacctgtattcgggcgcctggtgtcccctggcttcccagagaagtatgctgaccatcaagatcgatcctggacactgactgcaccccctggctaccgcctgcgcctctacttcacccactttgacctggaactctcttaccgctgcgagtatgactttgtcaagttgagctcagggaccaaggtgctggccacactgtgtgggcaggagagtacagacactgagcaggcacctggcaatgacaccttctactcactgggtcccagcctaaaggtcaccttccactccgactactccaatgagaagccgttcacagggtttgaggccttctatgcagcggaggatgtggatgaatgcagagtgtctctgggagactcagtcccttgtgaccattattgccacaactacttgggcggctactattgctcctgcagagcgggctacattctccaccagaacaagcacacgtgctcagccctttgttcaggccaggtgttcacaggaagatctgggtatctcagtagccctgagtacccgcagccataccccaagctctccagctgcacctacagcatccgcctggaggacggcttcagtgtcatcctggacttcgtggagtccttcgatgtggagacgcaccctgaagcccagtgcccctatgactccctcaagattcaaacagacaagggggaacacggcccattttgtgggaagacgctgcctcccaggattgaaactgacagccacaaggtgaccatcacctttgccactgacgagtcggggaaccacacaggctggaagatacactacacaagcacagcacggccctgccctgatccaacggcgccacctaatggcagcatttcacctgtgcaagccacgtatgtcctgaaggacaggttttctgtcttctgcaagacaggcttcgagcttctgcaaggttctgtccccctgaaatcattcactgctgtctgtcagaaagatggatcttgggaccggccgatgccagagtgcagcattattgattgtggccctcccgatgacctacccaatggccatgtggactatatcacaggccctcaagtgactacctacaaagctgtgattcagtacagctgtgaagagactttctacacaatgagcagcaatggtaaatatgtgtgtgaggctgatggattctggacgagctccaaaggagaaaaactccccccggtttgtgagcctgtttgtgggctgtccacacacactataggaggacgcatagttggagggcagcctgcaaagcctggtgactttccttggcaagtcttgttgctgggtcaaactacagcagcagcaggtgcacttatacatgacaattgggtcctaacagccgctcatgctgtatatgagaaaagaatggcagcgtcctccctgaacatccgaatgggcatcctcaaaaggctctcacctcattacactcaagcctggcccgaggaaatctttatacatgaaggctacactcacggtgctggttttgacaatgatatagcattgattaaactcaagaacaaagtcacaatcaacggaagcatcatgcctgtttgcctaccgcgaaaagaagctgcatccttaatgagaacagacttcactggaactgtggctggctgggggttaacccagaaggggcttcttgctagaaacctaatgtttgtggacataccaattgctgaccaccaaaaatgtaccaccgtgtatgaaaagctctatccaggagtaagagtaagcgctaacatgctctgtgctggcttagagactggtggcaaggacagctgcagaggtgacagtgggggggcattagtgtttctagataatgagacacagcgatggtttgtgggaggaatagtttcctggggttccattaattgtggggcggcaggccagtatggggtctacacaaaagtcatcaactatattccctggaatgagaacataataagtaatttctaa

SEQ ID NO: 51 - protein, 685 aa, Murine
MRLLIFLGLLWSLVATLLGSKWPEPVFGRLVSPGFPEKYADHQDRSWTLTAPPGYRLRLYFTHFDLELSYRCEYDFVKLSSGTKVLATLCGQESTDTEQAPGNDTFYSLGPSLKVTFHSDYSNEKPFTGFEAFYAAEDVDECRVSLGDSVPCDHYCHNYLGGYYCSCRAGYILHQNKHTCSALCSGQVFTGRSGYLSSPEYPQPYPKLSSCTYSIRLEDGFSVILDFVESFDVETHPEAQCPYDSLKIQTDKGEHGPFCGKTLPPRIETDSHKVTITFATDESGNHTGWKIHYTSTARPCPDPTAPPNGSISPVQATYVLKDRFSVFCKTGFELLQGSVPLKSFTAVCQKDGSWDRPMPECSIIDCGPPDDLPNGHVDYITGPQVTTYKAVIQYSCEETFYTMSSNGKYVCEADGFWTSSKGEKLPPVCEPVCGLSTHTIGGRIVGGQPAKPGDFPWQVLLLGQTTAAAGALIHDNWVLTAAHAVYEKRMAASSLNIRMGILKRLSPHYTQAWPEEIFIHEGYTHGAGFDNDIALIKLKNKVTINGSIMPVCLPRKEAASLMRTDFTGTVAGWGLTQKGLLARNLMFVDIPIADHQKCTTVYEKLYPGVRVSANMLCAGLETGGKDSCRGDSGGALVFLDNETQRWFVGGIVSWGSINCGAAGQYGVYTKVINYIPWNENIISNF

SEQ ID NO: 52 - protein, 670 aa, Murine
TLLGSKWPEPVFGRLVSPGFPEKYADHQDRSWTLTAPPGYRLRLYFTHFDLELSYRCEYDFVKLSSGTKVLATLCGQESTDTEQAPGNDTFYSLGPSLKVTFHSDYSNEKPFTGFEAFYAAEDVDECRVSLGDSVPCDHYCHNYLGGYYCSCRAGYILHQNKHTCSALCSGQVFTGRSGYLSSPEYPQPYPKLSSCTYSIRLEDGFSVILDFVESFDVETHPEAQCPYDSLKIQTDKGEHGPFCGKTLPPRIETDSHKVTITFATDESGNHTGWKIHYTSTARPCPDPTAPPNGSISPVQATYVLKDRFSVFCKTGFELLQGSVPLKSFTAVCQKDGSWDRPMPECSIIDCGPPDDLPNGHVDYITGPQVTTYKAVIQYSCEETFYTMSSNGKYVCEADGFWTSSKGEKLPPVCEPVCGLSTHTIGGRIVGGQPAKPGDFPWQVLLLGQTTAAAGALIHDNWVLTAAHAVYEKRMAASSLNIRMGILKRLSPHYTQAWPEEIFIHEGYTHGAGFDNDIALIKLKNKVTINGSIMPVCLPRKEAASLMRTDFTGTVAGWGLTQKGLLARNLMFVDIPIADHQKCTTVYEKLYPGVRVSANMLCAGLETGGKDSCRGDSGGALVFLDNETQRWFVGGIVSWGSINCGAAGQYGVYTKVINYIPWNENIISNF

SEQ ID NO: 53 - DNA, 2091 bp, Rat
  source 1..2091: mol_type = other DNA
tggcacacaatgaggctactgatcgtcctgggtctgctttggagtttggtggccacacttttgggctccaagtggcctgagcctgtattcgggcgcctggtgtccctggccttcccagagaagtatggcaaccatcaggatcgatcctggacgctgactgcaccccctggcttccgcctgcgcctctacttcacccacttcaacctggaactctcttaccgctgcgagtatgactttgtcaagttgacctcagggaccaaggtgctagccacgctgtgtgggcaggagagtacagatactgagcgggcacctggcaatgacaccttctactcactgggtcccagcctaaaggtcaccttccactccgactactccaatgagaagccattcacaggatttgaggccttctatgcagcggaggatgtggatgaatgcagaacatccctgggagactcagtcccttgtgaccattattgccacaactacctgggcggctactactgctcctgccgagtgggctacattctgcaccagaacaagcatacctgctcagccctttgttcaggccaggtgttcactgggaggtctggctttctcagtagccctgagtacccacagccataccccaaactctccagctgcgcctacaacatccgcctggaggaaggcttcagtatcaccctggacttcgtggagtcctttgatgtggagatgcaccctgaagcccagtgcccctacgactccctcaagattcaaacagacaagagggaatacggcccgttttgtgggaagacgctgccccccaggattgaaactgacagcaacaaggtgaccattacctttaccaccgacgagtcagggaaccacacaggctggaagatacactacacaagcacagcacagccctgccctgatccaacggcgccacctaatggtcacatttcacctgtgcaagccacgtatgtcctgaaggacagcttttctgtcttctgcaagactggcttcgagcttctgcaaggttctgtccccctgaagtcattcactgctgtctgtcagaaagatggatcttgggaccggccgataccagagtgcagcattattgactgtggccctcccgatgacctacccaatggccacgtggactatatcacaggccctgaagtgaccacctacaaagctgtgattcagtacagctgtgaagagactttctacacaatgagcagcaatggtaaatatgtgtgtgaggctgatggattctggacgagctccaaaggagaaaaatccctcccggtttgcaagcctgtctgtggactgtccacacacacttcaggaggccgtataattggaggacagcctgcaaagcctggtgactttccttggcaagtcttgttactgggtgaaactacagcagcaggtgctcttatacatgacgactgggtcctaacagcggctcatgctgtatatgggaaaacagaggcgatgtcctccctggacatccgcatgggcatcctcaaaaggctctccctcatttacactcaagcctggccagaggctgtctttatccatgaaggctacactcacggagctggttttgacaatgatatagcactgattaaactcaagaacaaagtcacaatcaacagaaacatcatgccgatttgtctaccaagaaaagaagctgcatccttaatgaaaacagacttcgttggaactgtggctggctgggggttaacccagaaggggtttcttgctagaaacctaatgtttgtggacataccaattgttgaccaccaaaaatgtgctactgcgtatacaaagcagccctacccaggagcaaaagtgactgttaacatgctctgtgctggcctagaccgcggtggcaaggacagctgcagaggtgacagcggaggggcattagtgtttctagacaatgaaacacagagatggtttgtgggaggaatagtttcctggggttctattaactgtggggggtcagaacagtatggggtctacacgaaagtcacgaactatattccctggattgagaacataataaataatttctaatttgcaaaaaaaaaaaaaaaaaaa

SEQ ID NO: 54 - protein, 685 aa, Rat
MRLLIVLGLLWSLVATLLGSKWPEPVFGRLVSLAFPEKYGNHQDRSWTLTAPPGFRLRLYFTHFNLELSYRCEYDFVKLTSGTKVLATLCGQESTDTERAPGNDTFYSLGPSLKVTFHSDYSNEKPFTGFEAFYAAEDVDECRTSLGDSVPCDHYCHNYLGGYYCSCRVGYILHQNKHTCSALCSGQVFTGRSGFLSSPEYPQPYPKLSSCAYNIRLEEGFSITLDFVESFDVEMHPEAQCPYDSLKIQTDKREYGPFCGKTLPPRIETDSNKVTITFTTDESGNHTGWKIHYTSTAQPCPDPTAPPNGHISPVQATYVLKDSFSVFCKTGFELLQGSVPLKSFTAVCQKDGSWDRPIPECSIIDCGPPDDLPNGHVDYITGPEVTTYKAVIQYSCEETFYTMSSNGKYVCEADGFWTSSKGEKSLPVCKPVCGLSTHTSGGRIIGGQPAKPGDFPWQVLLLGETTAAGALIHDDWVLTAAHAVYGKTEAMSSLDIRMGILKRLSLIYTQAWPEAVFIHEGYTHGAGFDNDIALIKLKNKVTINRNIMPICLPRKEAASLMKTDFVGTVAGWGLTQKGFLARNLMFVDIPIVDHQKCATAYTKQPYPGAKVTVNMLCAGLDRGGKDSCRGDSGGALVFLDNETQRWFVGGIVSWGSINCGGSEQYGVYTKVTNYIPWIENIINNF

SEQ ID NO: 55 - protein, 670 aa, Rat
TLLGSKWPEPVFGRLVSLAFPEKYGNHQDRSWTLTAPPGFRLRLYFTHFNLELSYRCEYDFVKLTSGTKVLATLCGQESTDTERAPGNDTFYSLGPSLKVTFHSDYSNEKPFTGFEAFYAAEDVDECRTSLGDSVPCDHYCHNYLGGYYCSCRVGYILHQNKHTCSALCSGQVFTGRSGFLSSPEYPQPYPKLSSCAYNIRLEEGFSITLDFVESFDVEMHPEAQCPYDSLKIQTDKREYGPFCGKTLPPRIETDSNKVTITFTTDESGNHTGWKIHYTSTAQPCPDPTAPPNGHISPVQATYVLKDSFSVFCKTGFELLQGSVPLKSFTAVCQKDGSWDRPIPECSIIDCGPPDDLPNGHVDYITGPEVTTYKAVIQYSCEETFYTMSSNGKYVCEADGFWTSSKGEKSLPVCKPVCGLSTHTSGGRIIGGQPAKPGDFPWQVLLLGETTAAGALIHDDWVLTAAHAVYGKTEAMSSLDIRMGILKRLSLIYTQAWPEAVFIHEGYTHGAGFDNDIALIKLKNKVTINRNIMPICLPRKEAASLMKTDFVGTVAGWGLTQKGFLARNLMFVDIPIVDHQKCATAYTKQPYPGAKVTVNMLCAGLDRGGKDSCRGDSGGALVFLDNETQRWFVGGIVSWGSINCGGSEQYGVYTKVTNYIPWIENIINNF

SEQ ID NO: 56 - DNA, 28 bp, synthetic construct
  misc_feature 1..28: note = Homo Sapiens
  source 1..28: mol_type = other DNA
atgaggctgctgaccctcctgggccttc

SEQ ID NO: 57 - DNA, 23 bp, synthetic construct
  misc_feature 1..23: note = Homo Sapiens
  source 1..23: mol_type = other DNA
gtgcccctcctgcgtcacctctg

SEQ ID NO: 58 - DNA, 23 bp, synthetic construct
  misc_feature 1..23: note = Homo Sapiens
  source 1..23: mol_type = other DNA
cagaggtgacgcaggaggggcac

SEQ ID NO: 59 - DNA, 27 bp, synthetic construct
  misc_feature 1..27: note = Homo Sapiens
  source 1..27: mol_type = other DNA
ttaaaatcactaattatgttctcgatc

SEQ ID NO: 60 - DNA, 22 bp, synthetic construct
  misc_feature 1..22: note = Murine
  source 1..22: mol_type = other DNA
atgaggctactcatcttcctgg

SEQ ID NO: 61 - DNA, 23 bp, synthetic construct
  misc_feature 1..23: note = Murine
  source 1..23: mol_type = other DNA
ctgcagaggtgacgcaggggggg

SEQ ID NO: 62 - DNA, 23 bp, synthetic construct
  misc_feature 1..23: note = Murine
  source 1..23: mol_type = other DNA
ccccccctgcgtcacctctgcag

SEQ ID NO: 63 - DNA, 29 bp, synthetic construct
  misc_feature 1..29: note = Murine
  source 1..29: mol_type = other DNA
ttagaaattacttattatgttctcaatcc

SEQ ID NO: 64 - DNA, 29 bp, synthetic construct
  misc_feature 1..29: note = Rat
  source 1..29: mol_type = other DNA
gaggtgacgcaggaggggcattagtgttt

SEQ ID NO: 65 - DNA, 37 bp, synthetic construct
  misc_feature 1..37: note = Rat
  source 1..37: mol_type = other DNA
ctagaaacactaatgcccctcctgcgtcacctctgca

SEQ ID NO: 66 - DNA, 354 bp, synthetic construct
  misc_feature 1..354: note = Synthetic
  source 1..354: mol_type = other DNA
caggtcaccttgaaggagtctggtcctgtgctggtgaaacccacagagaccctcacgctgacctgcaccgtctctgggttctcactcagcaggggtaaaatgggtgtgagctggatccgtcagcccccagggaaggccctggagtggcttgcacacattttttcgagtgacgaaaaatcctacaggacatcgctgaagagcaggctcaccatctccaaggacacctccaaaaaccaggtggtccttacaatgaccaacatggaccctgtggacacagccacgtattactgtgcacggatacgacgtggaggaattgactactggggccagggaaccctggtcactgtctcctca

SEQ ID NO: 67 - protein, 118 aa, synthetic construct
  REGION 1..118: note = Synthetic
QVTLKESGPVLVKPTETLTLTCTVSGFSLSRGKMGVSWIRQPPGKALEWLAHIFSSDEKSYRTSLKSRLTISKDTSKNQVVLTMTNMDPVDTATYYCARIRRGGIDYWGQGTLVTVSS

SEQ ID NO: 68 - protein, 121 aa, synthetic construct
  REGION 1..121: note = Synthetic
QVQLQQSGPGLVKPSQTLSLTCAISGDSVSSTSAAWNWIRQSPSRGLEWLGRTYYRSKWYNDYAVSVKSRITINPDTSKNQFSLQLNSVTPEDTAVYYCARDPFGVPFDIWGQGTMVTVSS

SEQ ID NO: 69 - protein, 106 aa, synthetic construct
  REGION 1..106: note = Synthetic
QPVLTQPPSLSVSPGQTASITCSGEKLGDKYAYWYQQKPGQSPVLVMYQDKQRPSGIPERFSGSNSGNTATLTISGTQAMDEADYYCQAWDSSTAVFGGGTKLTVL

SEQ ID NO: 70 - DNA, 324 bp, synthetic construct
  misc_feature 1..324: note = Synthetic
  source 1..324: mol_type = other DNA
tcctatgagctgatacagccaccctcggtgtcagtggccccaggacagacggccaccattacctgtgcgggagacaaccttgggaagaaacgtgtgcactggtaccagcagaggccaggccaggcccctgtgttggtcatctatgatgatagcgaccggccctcagggatccctgaccgattctctgcctccaactctgggaacacggccaccctgaccatcactaggggcgaagccggggatgaggccgactattattgtcaggtgtgggacattgctactgatcatgtggtcttcggcggagggaccaagctcaccgtccta

SEQ ID NO: 71 - protein, 120 aa, synthetic construct
  REGION 1..120: note = Synthetic
SYELIQPPSVSVAPGQTATITCAGDNLGKKRVHWYQQRPGQAPVLVIYDDSDRPSGIPDRFSASNSGNTATLTITRGEAGDEADYYCQVWDIATDHVVFGGGTKLTVLAAAGSEQKLISE

SEQ ID NO: 72 - protein, 36 aa, synthetic construct
  REGION 1..36: note = Synthetic
LEVTCEPGTTFKDKCNTCRCGSDGKSAVCTKLWCNQ

SEQ ID NO: 73 - protein, 33 aa, synthetic construct
  REGION 1..33: note = Synthetic
TCEPGTTFKDKCNTCRCGSDGKSAVCTKLWCNQ

SEQ ID NO: 74 - protein, 20 aa, synthetic construct
  REGION 1..20: note = Synthetic
TCRCGSDGKSAVCTKLWCNQ

SEQ ID NO: 75 - protein, 491 aa, synthetic construct
  REGION 1..491: note = Synthetic
LEVTCEPGTTFKDKCNTCRCGSDGKSAVCTKLWCNQGTGGGSGSSSQVTLKESGPVLVKPTETLTLTCTVSGFSLSRGKMGVSWIRQPPGKALEWLAHIFSSDEKSYRTSLKSRLTISKDTSKNQVVLTMTNMDPVDTATYYCARIRRGGIDYWGQGTLVTVSSASTKGPSVFPLAPCSRSTSESTAALGCLVKDYFPEPVTVSWNSGALTSGVHTFPAVLQSSGLYSLSSVVTVPSSSLGTKTYTCNVDHKPSNTKVDKRVESKYGPPCPPCPAPEFLGGPSVFLFPPKPKDTLMISRTPEVTCVVVDVSQEDPEVQFNWYVDGVEVHNAKTKPREEQFNSTYRVVSVLTVLHQDWLNGKEYKCKVSNKGLPSSIEKTISKAKGQPREPQVYTLPPSQEEMTKNQVSLTCLVKGFYPSDIAVEWESNGQPENNYKTTPPVLDSDGSFFLYSRLTVDKSRWQEGNVFSCSVMHEALHNHYTQKSLSLSLGK

SEQ ID NO: 76 - protein, 491 aa, synthetic construct
  REGION 1..491: note = Synthetic
QVTLKESGPVLVKPTETLTLTCTVSGFSLSRGKMGVSWIRQPPGKALEWLAHIFSSDEKSYRTSLKSRLTISKDTSKNQVVLTMTNMDPVDTATYYCARIRRGGIDYWGQGTLVTVSSASTKGPSVFPLAPCSRSTSESTAALGCLVKDYFPEPVTVSWNSGALTSGVHTFPAVLQSSGLYSLSSVVTVPSSSLGTKTYTCNVDHKPSNTKVDKRVESKYGPPCPPCPAPEFLGGPSVFLFPPKPKDTLMISRTPEVTCVVVDVSQEDPEVQFNWYVDGVEVHNAKTKPREEQFNSTYRVVSVLTVLHQDWLNGKEYKCKVSNKGLPSSIEKTISKAKGQPREPQVYTLPPSQEEMTKNQVSLTCLVKGFYPSDIAVEWESNGQPENNYKTTPPVLDSDGSFFLYSRLTVDKSRWQEGNVFSCSVMHEALHNHYTQKSLSLSLGKAAGGSGLEVTCEPGTTFKDKCNTCRCGSDGKSAVCTKLWCNQGSGA

SEQ ID NO: 77 - protein, 258 aa, synthetic construct
  REGION 1..258: note = Synthetic
LEVTCEPGTTFKDKCNTCRCGSDGKSAVCTKLWCNQGTGGGSGSSSQPVLTQPPSLSVSPGQTASITCSGEKLGDKYAYWYQQKPGQSPVLVMYQDKQRPSGIPERFSGSNSGNTATLTISGTQAMDEADYYCQAWDSSTAVFGGGTKLTVLGQPKAAPSVTLFPPSSEELQANKATLVCLISDFYPGAVTVAWKADSSPVKAGVETTTPSKQSNNKYAASSYLSLTPEQWKSHRSYSCQVTHEGSTVEKTVAPTECS

SEQ ID NO: 78 - protein, 258 aa, synthetic construct
  REGION 1..258: note = Synthetic
QPVLTQPPSLSVSPGQTASITCSGEKLGDKYAYWYQQKPGQSPVLVMYQDKQRPSGIPERFSGSNSGNTATLTISGTQAMDEADYYCQAWDSSTAVFGGGTKLTVLGQPKAAPSVTLFPPSSEELQANKATLVCLISDFYPGAVTVAWKADSSPVKAGVETTTPSKQSNNKYAASSYLSLTPEQWKSHRSYSCQVTHEGSTVEKTVAPTECSAAGGSGLEVTCEPGTTFKDKCNTCRCGSDGKSAVCTKLWCNQGSGA

SEQ ID NO: 79 - protein, 10 aa, synthetic construct
  REGION 1..10: note = Synthetic
GTGGGSGSSS

SEQ ID NO: 80 - protein, 6 aa, synthetic construct
  REGION 1..6: note = Synthetic
AAGGSG

SEQ ID NO: 81 - protein, 4 aa, synthetic construct
  REGION 1..4: note = Synthetic
GSGA

SEQ ID NO: 82 - DNA, 1533 bp, synthetic construct
  misc_feature 1..1533: note = Synthetic
  source 1..1533: mol_type = other DNA
atgatgtcctttgtctctctgctcctggttggcatcctattccatgccacccaggccttggaagtgacgtgtgagcccggaacgacattcaaagacaagtgcaatacttgtcggtgcggttcagatgggaaatcggcggtctgcacaaagctctggtgtaaccagggcaccggtggagggtcgggatccagctcacaggtcaccttgaaggagtctggtcctgtgctggtgaaacccacagagaccctcacgctgacctgcaccgtctctgggttctcactcagcaggggtaaaatgggtgtgagctggatccgtcagcccccagggaaggccctggagtggcttgcacacattttttcgagtgacgaaaaatcctacaggacatcgctgaagagcaggctcaccatctccaaggacacctccaaaaaccaggtggtccttacaatgaccaacatggaccctgtggacacagccacgtattactgtgcacggatacgacgtggaggaattgactactggggccagggaaccctggtcactgtctcctcagcctccaccaagggcccatccgtcttccccctggcgccctgctccaggagcacctccgagagcacagccgccctgggctgcctggtcaaggactacttccccgaaccggtgacggtgtcgtggaactcaggcgccctgaccagcggcgtgcacaccttcccggctgtcctacagtcctcaggactctactccctcagcagcgtggtgaccgtgccctccagcagcttgggcacgaagacctacacctgcaacgtagatcacaagcccagcaacaccaaggtggacaagagagttgagtccaaatatggtcccccatgcccaccatgcccagcacctgagttcctggggggaccatcagtcttcctgttccccccaaaacccaaggacactctcatgatctcccggacccctgaggtcacgtgcgtggtggtggacgtgagccaggaagaccccgaggtccagttcaactggtacgtggatggcgtggaggtgcataatgccaagacaaagccgcgggaggagcagttcaacagcacgtaccgtgtggtcagcgtcctcaccgtcctgcaccaggactggctgaacggcaaggagtacaagtgcaaggtctccaacaaaggcctcccgtcctccatcgagaaaaccatctccaaagccaaagggcagccccgagagccacaggtgtacaccctgcccccatcccaggaggagatgaccaagaaccaggtcagcctgacctgcctggtcaaaggcttctaccccagcgacatcgccgtggagtgggagagcaatgggcagccggagaacaactacaagaccacgcctcccgtgctggactccgacggctccttcttcctctacagcaggctaaccgtggacaagagcaggtggcaggaggggaatgtcttctcatgctccgtgatgcatgaggctctgcacaaccactacacacagaagagcctctccctgtctctcgggaaatga

SEQ ID NO: 83 - DNA, 1533 bp, synthetic construct
  misc_feature 1..1533: note = Synthetic
  source 1..1533: mol_type = other DNA
atgatgtcctttgtctctctgctcctggttggcatcctattccatgccacccaggcccaggtcaccttgaaggagtctggtcctgtgctggtgaaacccacagagaccctcacgctgacctgcaccgtctctgggttctcactcagcaggggtaaaatgggtgtgagctggatccgtcagcccccagggaaggccctggagtggcttgcacacattttttcgagtgacgaaaaatcctacaggacatcgctgaagagcaggctcaccatctccaaggacacctccaaaaaccaggtggtccttacaatgaccaacatggaccctgtggacacagccacgtattactgtgcacggatacgacgtggaggaattgactactggggccagggaaccctggtcactgtctcctcagcctccaccaagggcccatccgtcttccccctggcgccctgctccaggagcacctccgagagcacagccgccctgggctgcctggtcaaggactacttccccgaaccggtgacggtgtcgtggaactcaggcgccctgaccagcggcgtgcacaccttcccggctgtcctacagtcctcaggactctactccctcagcagcgtggtgaccgtgccctccagcagcttgggcacgaagacctacacctgcaacgtagatcacaagcccagcaacaccaaggtggacaagagagttgagtccaaatatggtcccccatgcccaccatgcccagcacctgagttcctggggggaccatcagtcttcctgttccccccaaaacccaaggacactctcatgatctcccggacccctgaggtcacgtgcgtggtggtggacgtgagccaggaagaccccgaggtccagttcaactggtacgtggatggcgtggaggtgcataatgccaagacaaagccgcgggaggagcagttcaacagcacgtaccgtgtggtcagcgtcctcaccgtcctgcaccaggactggctgaacggcaaggagtacaagtgcaaggtctccaacaaaggcctcccgtcctccatcgagaaaaccatctccaaagccaaagggcagccccgagagccacaggtgtacaccctgcccccatcccaggaggagatgaccaagaaccaggtcagcctgacctgcctggtcaaaggcttctaccccagcgacatcgccgtggagtgggagagcaatgggcagccggagaacaactacaagaccacgcctcccgtgctggactccgacggctccttcttcctctacagcaggctaaccgtggacaagagcaggtggcaggaggggaatgtcttctcatgctccgtgatgcatgaggctctgcacaaccactacacacagaagagcctctccctgtctctcgggaaagccgctggtggtagtggtttggaagtgacgtgtgagcccggaacgacattcaaagacaagtgcaatacttgtcggtgcggttcagatgggaaatcggcggtctgcacaaagctctggtgtaaccagggtagtggtgcttga

SEQ ID NO: 84 - DNA, 834 bp, synthetic construct
  misc_feature 1..834: note = Synthetic
  source 1..834: mol_type = other DNA
atgatgtcctttgtctctctgctcctggttggcatcctattccatgccacccaggccttggaagtgacgtgtgagcccggaacgacattcaaagacaagtgcaatacttgtcggtgcggttcagatgggaaatcggcggtctgcacaaagctctggtgtaaccagggcaccggtggagggtcgggatccagctcacagccagtgctgactcagcccccctcactgtccgtgtccccaggacagacagccagcatcacctgctctggagagaaattgggggataaatatgcttactggtatcagcagaagccaggccagtcccctgtgttggtcatgtatcaagataaacagcggccctcagggatccctgagcgattctctggctccaactctgggaacacagccactctgaccatcagcgggacccaggctatggatgaggctgactattactgtcaggcgtgggacagcagcactgcggtattcggcggagggaccaagctgaccgtcctaggccagcctaaggcggcgccctcggtcaccctgttcccgccctcctctgaggagcttcaagccaacaaggccacactggtgtgtctcataagtgacttctacccgggagccgtgacagtggcctggaaggcagatagcagccccgtcaaggcgggagtggagaccaccacaccctccaaacaaagcaacaacaagtacgcggccagcagctatctgagcctgacgcctgagcagtggaagtcccacagaagctacagctgccaggtcacgcatgaagggagcaccgtggagaagacagtggcccctacagaatgttcatag

SEQ ID NO: 85 - DNA, 834 bp, synthetic construct
  misc_feature 1..834: note = Synthetic
  source 1..834: mol_type = other DNA
atgatgtcctttgtctctctgctcctggttggcatcctattccatgccacccaggcccagccagtgctgactcagcccccctcactgtccgtgtccccaggacagacagccagcatcacctgctctggagagaaattgggggataaatatgcttactggtatcagcagaagccaggccagtcccctgtgttggtcatgtatcaagataaacagcggccctcagggatccctgagcgattctctggctccaactctgggaacacagccactctgaccatcagcgggacccaggctatggatgaggctgactattactgtcaggcgtgggacagcagcactgcggtattcggcggagggaccaagctgaccgtcctaggccagcctaaggcggcgccctcggtcaccctgttcccgccctcctctgaggagcttcaagccaacaaggccacactggtgtgtctcataagtgacttctacccgggagccgtgacagtggcctggaaggcagatagcagccccgtcaaggcgggagtggagaccaccacaccctccaaacaaagcaacaacaagtacgcggccagcagctatctgagcctgacgcctgagcagtggaagtcccacagaagctacagctgccaggtcacgcatgaagggagcaccgtggagaagacagtggcccctacagaatgttcagccgctggtggtagtggtttggaagtgacgtgtgagcccggaacgacattcaaagacaagtgcaatacttgtcggtgcggttcagatgggaaatcggcggtctgcacaaagctctggtgtaaccagggtagtggtgcttag